European Patent Specification EP 4 511 510 B1, published December 10, 2025. Title: AP50 POLYMERASES AND USES THEREOF. Applicant: 10x Genomics, Inc. Application WO. The sequence listing filed with the application follows.

SEQUENCE LISTING (38 sequences)

SEQ ID NO: 1 - protein, 731 aa, Synthetic construct
  REGION 1..731: note = APol (aa) without initial Met
GSNKQKKERQKPAKLLTLDTETRGLTGNVFRVGLFDGTNYYKSNTFDEILDLFEQYKDYECHVYVHNLDFDLAKIATTLFKRDRVRFAKSIFINGNVVTLHSDSMILHDSLRLLPGSLEKLCKDFGLTDNAKKDLSEVIKEQGYAVYKKDGVTFDKKKSLGNYFENVPADDPTLNEYLEFDCRSLYEILTIVMDIANIGLETLVMCPTTASLAMRVYKEQYREQYDKVATHFYMGEWGQFLEEHVRQSYYGGRTEVFTPHLPHGYHYDVNSLYPYVMKIAKFPVGYPNLLKDGQAATKWKHWKRRAIGGGVMWCRVDVPEDMYIPVLPKRDPSGKLLFPVGKLEGVWTLPELLEAEKNGCTIEAIYQMVYWEHMEPIFKEFVEHFEDLKKNSKGAKRTFAKLIQNSLYGKFGMNRVRVSLGDMEDRYDLHEKQIPYKEFKHDCNGLTLEFIQYISESKASYIQPHIATYVTAYARILLFRGLKEQASKGVLGYCDTDSIAGTAKMPDEMIHDEDYGKWALEGELEEGIFLQPKFYAERYTNGKEVIKAKGIPREKMEELSFENYKEWLEIMKEGQQERIDIFEGYESRKKFSTTLKASEDFDTLREMKKSINLLLEQKRDIDYKGNVTRPHKRYDYGDKKDKIDYEDYKSREDKLNNMYDDVDDLKEQVDEIGYIKCMKQGDMYFEEYKHLTKSVKSKYFRRTGTPIDVWANESGWDVNELLEELRLMGVC

SEQ ID NO: 2 - protein, 740 aa, Synthetic construct
  REGION 1..740: note = APol-His (aa) without initial Met
GSNKQKKERQKPAKLLTLDTETRGLTGNVFRVGLFDGTNYYKSNTFDEILDLFEQYKDYECHVYVHNLDFDLAKIATTLFKRDRVRFAKSIFINGNVVTLHSDSMILHDSLRLLPGSLEKLCKDFGLTDNAKKDLSEVIKEQGYAVYKKDGVTFDKKKSLGNYFENVPADDPTLNEYLEFDCRSLYEILTIVMDIANIGLETLVMCPTTASLAMRVYKEQYREQYDKVATHFYMGEWGQFLEEHVRQSYYGGRTEVFTPHLPHGYHYDVNSLYPYVMKIAKFPVGYPNLLKDGQAATKWKHWKRRAIGGGVMWCRVDVPEDMYIPVLPKRDPSGKLLFPVGKLEGVWTLPELLEAEKNGCTIEAIYQMVYWEHMEPIFKEFVEHFEDLKKNSKGAKRTFAKLIQNSLYGKFGMNRVRVSLGDMEDRYDLHEKQIPYKEFKHDCNGLTLEFIQYISESKASYIQPHIATYVTAYARILLFRGLKEQASKGVLGYCDTDSIAGTAKMPDEMIHDEDYGKWALEGELEEGIFLQPKFYAERYTNGKEVIKAKGIPREKMEELSFENYKEWLEIMKEGQQERIDIFEGYESRKKFSTTLKASEDFDTLREMKKSINLLLEQKRDIDYKGNVTRPHKRYDYGDKKDKIDYEDYKSREDKLNNMYDDVDDLKEQVDEIGYIKCMKQGDMYFEEYKHLTKSVKSKYFRRTGTPIDVWANESGWDVNELLEELRLMGVCGGSHHHHHH

SEQ ID NO: 3 - protein, 646 aa, Synthetic construct
  REGION 1..646: note = APolTr-His (aa) without initial Met
GSNKQKKERQKPAKLLTLDTETRGLTGNVFRVGLFDGTNYYKSNTFDEILDLFEQYKDYECHVYVHNLDFDLAKIATTLFKRDRVRFAKSIFINGNVVTLHSDSMILHDSLRLLPGSLEKLCKDFGLTDNAKKDLSEVIKEQGYAVYKKDGVTFDKKKSLGNYFENVPADDPTLNEYLEFDCRSLYEILTIVMDIANIGLETLVMCPTTASLAMRVYKEQYREQYDKVATHFYMGEWGQFLEEHVRQSYYGGRTEVFTPHLPHGYHYDVNSLYPYVMKIAKFPVGYPNLLKDGQAATKWKHWKRRAIGGGVMWCRVDVPEDMYIPVLPKRDPSGKLLFPVGKLEGVWTLPELLEAEKNGCTIEAIYQMVYWEHMEPIFKEFVEHFEDLKKNSKGAKRTFAKLIQNSLYGKFGMNRVRVSLGDMEDRYDLHEKQIPYKEFKHDCNGLTLEFIQYISESKASYIQPHIATYVTAYARILLFRGLKEQASKGVLGYCDTDSIAGTAKMPDEMIHDEDYGKWALEGELEEGIFLQPKFYAERYTNGKEVIKAKGIPREKMEELSFENYKEWLEIMKEGQQERIDIFEGYESRKKFSTTLKASEDFDTLREMKKSINLLLEQKRDIDYKGNVTRPHKRYDYGGGSHHHHHH

SEQ ID NO: 4 - protein, 657 aa, Synthetic construct
  REGION 1..657: note = APolTr-His-SET (aa) without initial Met
GSNKQKKERQKPAKLLTLDTETRGLTGNVFRVGLFDGTNYYKSNTFDEILDLFEQYKDYECHVYVHNLDFDLAKIATTLFKRDRVRFAKSIFINGNVVTLHSDSMILHDSLRLLPGSLEKLCKDFGLTDNAKKDLSEVIKEQGYAVYKKDGVTFDKKKSLGNYFENVPADDPTLNEYLEFDCRSLYEILTIVMDIANIGLETLVMCPTTASLAMRVYKEQYREQYDKVATHFYMGEWGQFLEEHVRQSYYGGRTEVFTPHLPHGYHYDVNSLYPYVMKIAKFPVGYPNLLKDGQAATKWKHWKRRAIGGGVMWCRVDVPEDMYIPVLPKRDPSGKLLFPVGKLEGVWTLPELLEAEKNGCTIEAIYQMVYWEHMEPIFKEFVEHFEDLKKNSKGAKRTFAKLIQNSLYGKFGMNRVRVSLGDMEDRYDLHEKQIPYKEFKHDCNGLTLEFIQYISESKASYIQPHIATYVTAYARILLFRGLKEQASKGVLGYCDTDSIAGTAKMPDEMIHDEDYGKWALEGELEEGIFLQPKFYAERYTNGKEVIKAKGIPREKMEELSFENYKEWLEIMKEGQQERIDIFEGYESRKKFSTTLKASEDFDTLREMKKSINLLLEQKRDIDYKGNVTRPHKRYDYGGGSHHHHHHSEEDEEKEEDG

SEQ ID NO: 5 - protein, 574 aa, Synthetic construct
  REGION 1..574: note = Phi29 WT (aa) without initial Met
KHMPRKMYSCDFETTTKVEDCRVWAYGYMNIEDHSEYKIGNSLDEFMAWVLKVQADLYFHNLKFDGAFIINWLERNGFKWSADGLPNTYNTIISRMGQWYMIDICLGYKGKRKIHTVIYDSLKKLPFPVKKIAKDFKLTVLKGDIDYHKERPVGYKITPEEYAYIKNDIQIIAEALLIQFKQGLDRMTAGSDSLKGFKDIITTKKFKKVFPTLSLGLDKEVRYAYRGGFTWLNDRFKEKEIGEGMVFDVNSLYPAQMYSRLLPYGEPIVFEGKYVWDEDYPLHIQHIRCEFELKEGYIPTIQIKRSRFYKGNEYLKSSGGEIADLWLSNVDLELMKEHYDLYNVEYISGLKFKATTGLFKDFIDKWTYIKTTSEGAIKQLAKLMLNSLYGKFASNPDVTGKVPYLKENGALGFRLGEEETKDPVYTPMGVFITAWARYTTITAAQACYDRIIYCDTDSIHLTGTEIPDVIKDIVDPKKLGYWAHESTFKRAKYLRQKTYIQDIYMKEVDGKLVEGSPDDYTDIKFSVKCAGMTDKIKKEVTFENFKVGFSRKMKPKPVQVPGGVVLVDDTFTIK

SEQ ID NO: 6 - protein, 637 aa, Synthetic construct
  REGION 1..637: note = APolTr (aa) without initial Met
GSNKQKKERQKPAKLLTLDTETRGLTGNVFRVGLFDGTNYYKSNTFDEILDLFEQYKDYECHVYVHNLDFDLAKIATTLFKRDRVRFAKSIFINGNVVTLHSDSMILHDSLRLLPGSLEKLCKDFGLTDNAKKDLSEVIKEQGYAVYKKDGVTFDKKKSLGNYFENVPADDPTLNEYLEFDCRSLYEILTIVMDIANIGLETLVMCPTTASLAMRVYKEQYREQYDKVATHFYMGEWGQFLEEHVRQSYYGGRTEVFTPHLPHGYHYDVNSLYPYVMKIAKFPVGYPNLLKDGQAATKWKHWKRRAIGGGVMWCRVDVPEDMYIPVLPKRDPSGKLLFPVGKLEGVWTLPELLEAEKNGCTIEAIYQMVYWEHMEPIFKEFVEHFEDLKKNSKGAKRTFAKLIQNSLYGKFGMNRVRVSLGDMEDRYDLHEKQIPYKEFKHDCNGLTLEFIQYISESKASYIQPHIATYVTAYARILLFRGLKEQASKGVLGYCDTDSIAGTAKMPDEMIHDEDYGKWALEGELEEGIFLQPKFYAERYTNGKEVIKAKGIPREKMEELSFENYKEWLEIMKEGQQERIDIFEGYESRKKFSTTLKASEDFDTLREMKKSINLLLEQKRDIDYKGNVTRPHKRYDYG

SEQ ID NO: 7 - protein, 6 aa, Synthetic construct
  REGION 1..6: note = 6x His tag (aa)
HHHHHH

SEQ ID NO: 8 - protein, 11 aa, Synthetic construct
  REGION 1..11: note = Solubility enhancement tag (SET)(aa)
SEEDEEKEEDG

SEQ ID NO: 9 - protein, 20 aa, Synthetic construct
  REGION 1..20: note = GSS linker-6x His-SET (aa)
GGSHHHHHHSEEDEEKEEDG

SEQ ID NO: 10 - skipped

SEQ ID NO: 11 - protein, 5 aa, Synthetic construct
  REGION 1..5: note = GGSGG linker (aa)
GGSGG

SEQ ID NO: 12 - protein, 5 aa, Synthetic construct
  REGION 1..5: note = GGGGG linker (aa)
GGGGG

SEQ ID NO: 13 - protein, 5 aa, Synthetic construct
  REGION 1..5: note = GGAGG linker (aa)
GGAGG

SEQ ID NO: 14 - protein, 7 aa, Synthetic construct
  REGION 1..7: note = GGGGSSS linker (aa)
GGGGSSS

SEQ ID NO: 15 - protein, 7 aa, Synthetic construct
  REGION 1..7: note = GGGGAAA linker (aa)
GGGGAAA

SEQ ID NO: 16 - protein, 50 aa, Synthetic construct
  REGION 1..50: note = GGGGS linker
  VARIANT 5..50: note = may be absent
GGGGSGGGGSGGGGSGGGGSGGGGSGGGGSGGGGSGGGGSGGGGSGGGGS

SEQ ID NO: 17 - DNA, 2193 bp, Synthetic construct
  misc_feature 1..2193: note = APol (nt)
  source 1..2193: mol_type = other DNA
ggctccaataagcaaaagaaagagcgccaaaagccggccaagcttctcaccttggacactgagacgcgcggcctcaccggtaatgtgttccgcgttggcctgtttgacgggacgaattattacaagtcgaatacattcgacgagatccttgacctgttcgagcaatataaagattacgaatgtcatgtatacgtacacaatttagacttcgacttggcgaaaatcgccaccactttgttcaagcgcgaccgtgtgcgctttgcgaagagcatcttcattaacggtaacgtagtgactttgcattcggactcgatgatcttacatgatagcttacgcttactgccggggtctctggaaaagctctgtaaagattttggcctgaccgacaacgccaagaaagatctttccgaagtcatcaaagagcagggttacgcagtatacaagaaagacggtgtcacatttgacaagaagaaatcccttggcaattattttgagaacgtgcctgccgacgaccctacgctcaatgagtacttggagttcgattgtcgcagcctgtacgagattttgacgattgtgatggacatcgcaaatattggcctggaaaccttagtaatgtgcccgaccacagcgagcttagccatgcgtgtctataaagagcaataccgcgagcaatatgataaggtggccactcacttttatatgggcgagtggggtcaattcctcgaagagcacgttcgccaatcgtactacggtggtcgcactgaggtatttacccctcatttaccacatggttaccattacgatgttaactcgttgtacccgtatgtcatgaaaattgcaaagttcccggtagggtacccaaatttattgaaagacggccaggcagctaccaagtggaagcattggaagcgtcgtgcgatcgggggcggtgttatgtggtgtcgtgtggacgttcctgaagacatgtacatcccagtgctcccgaagcgtgacccgagcgggaagttattgttcccggttggtaagctcgagggagtgtggaccctgcctgagctcctggaagcggaaaagaatggctgtacgatcgaggcgatttaccagatggtatactgggagcatatggagccgatctttaaagaattcgttgagcactttgaagacctcaagaagaacagtaagggagcgaagcgcacctttgcaaagcttatccagaatagcttgtacgggaagttcggcatgaaccgcgttcgtgtgtcgttgggtgacatggaagaccgttacgacttgcatgagaagcagattccatataaagaattcaaacatgattgtaatggcttgacgcttgagttcatccaatatatctcggaaagcaaagcgagctatattcaaccgcacattgctacatacgtaacagcctatgctcgtatcctgttgtttcgtggtctgaaagaacaggctagcaagggcgtactgggctattgcgatactgactctattgccggtaccgccaaaatgccggacgaaatgatccatgacgaagattacggcaagtgggccttggaaggtgagctggaagaaggtatctttctccagccgaagttttacgcggaacgttacacgaacggcaaagaagtaattaaggccaaggggattccacgcgagaagatggaagagttaagtttcgagaactataaagagtggctcgagattatgaaagaaggccaacaagagcgcatcgacatctttgaaggttacgagagtcgcaagaagtttagcaccacactcaaggccagtgaagatttcgacacgttgcgtgagatgaagaagtctatcaatttactgctcgagcagaagcgcgacatcgactacaagggcaacgtgacacgtccacataagcgctatgactacggtgataagaaagacaagatcgattatgaagactataagagccgtgaagacaagttaaacaacatgtacgacgatgtagacgacttaaaagagcaagttgacgagatcggctacatcaagtgcatgaagcaaggcgatatgtattttgaagagtacaaacatcttacgaagtctgtgaaaagtaagtatttccgccgcactggcaccccaatcgacgtatgggcgaacgaatccggttgggacgtaaacgagttattagaagagcttcgtctgatgggcgtgtgc

SEQ ID NO: 18 - DNA, 2220 bp, Synthetic construct
  misc_feature 1..2220: note = APol-His (nt)
  source 1..2220: mol_type = other DNA
ggctccaataagcaaaagaaagagcgccaaaagccggccaagcttctcaccttggacactgagacgcgcggcctcaccggtaatgtgttccgcgttggcctgtttgacgggacgaattattacaagtcgaatacattcgacgagatccttgacctgttcgagcaatataaagattacgaatgtcatgtatacgtacacaatttagacttcgacttggcgaaaatcgccaccactttgttcaagcgcgaccgtgtgcgctttgcgaagagcatcttcattaacggtaacgtagtgactttgcattcggactcgatgatcttacatgatagcttacgcttactgccggggtctctggaaaagctctgtaaagattttggcctgaccgacaacgccaagaaagatctttccgaagtcatcaaagagcagggttacgcagtatacaagaaagacggtgtcacatttgacaagaagaaatcccttggcaattattttgagaacgtgcctgccgacgaccctacgctcaatgagtacttggagttcgattgtcgcagcctgtacgagattttgacgattgtgatggacatcgcaaatattggcctggaaaccttagtaatgtgcccgaccacagcgagcttagccatgcgtgtctataaagagcaataccgcgagcaatatgataaggtggccactcacttttatatgggcgagtggggtcaattcctcgaagagcacgttcgccaatcgtactacggtggtcgcactgaggtatttacccctcatttaccacatggttaccattacgatgttaactcgttgtacccgtatgtcatgaaaattgcaaagttcccggtagggtacccaaatttattgaaagacggccaggcagctaccaagtggaagcattggaagcgtcgtgcgatcgggggcggtgttatgtggtgtcgtgtggacgttcctgaagacatgtacatcccagtgctcccgaagcgtgacccgagcgggaagttattgttcccggttggtaagctcgagggagtgtggaccctgcctgagctcctggaagcggaaaagaatggctgtacgatcgaggcgatttaccagatggtatactgggagcatatggagccgatctttaaagaattcgttgagcactttgaagacctcaagaagaacagtaagggagcgaagcgcacctttgcaaagcttatccagaatagcttgtacgggaagttcggcatgaaccgcgttcgtgtgtcgttgggtgacatggaagaccgttacgacttgcatgagaagcagattccatataaagaattcaaacatgattgtaatggcttgacgcttgagttcatccaatatatctcggaaagcaaagcgagctatattcaaccgcacattgctacatacgtaacagcctatgctcgtatcctgttgtttcgtggtctgaaagaacaggctagcaagggcgtactgggctattgcgatactgactctattgccggtaccgccaaaatgccggacgaaatgatccatgacgaagattacggcaagtgggccttggaaggtgagctggaagaaggtatctttctccagccgaagttttacgcggaacgttacacgaacggcaaagaagtaattaaggccaaggggattccacgcgagaagatggaagagttaagtttcgagaactataaagagtggctcgagattatgaaagaaggccaacaagagcgcatcgacatctttgaaggttacgagagtcgcaagaagtttagcaccacactcaaggccagtgaagatttcgacacgttgcgtgagatgaagaagtctatcaatttactgctcgagcagaagcgcgacatcgactacaagggcaacgtgacacgtccacataagcgctatgactacggtgataagaaagacaagatcgattatgaagactataagagccgtgaagacaagttaaacaacatgtacgacgatgtagacgacttaaaagagcaagttgacgagatcggctacatcaagtgcatgaagcaaggcgatatgtattttgaagagtacaaacatcttacgaagtctgtgaaaagtaagtatttccgccgcactggcaccccaatcgacgtatgggcgaacgaatccggttgggacgtaaacgagttattagaagagcttcgtctgatgggcgtgtgcggtggctcacatcaccaccatcatcat

SEQ ID NO: 19 - DNA, 1938 bp, Synthetic construct
  misc_feature 1..1938: note = APolTr-His (nt)
  source 1..1938: mol_type = other DNA
ggctccaataagcaaaagaaagagcgccaaaagccggccaagcttctcaccttggacactgagacgcgcggcctcaccggtaatgtgttccgcgttggcctgtttgacgggacgaattattacaagtcgaatacattcgacgagatccttgacctgttcgagcaatataaagattacgaatgtcatgtatacgtacacaatttagacttcgacttggcgaaaatcgccaccactttgttcaagcgcgaccgtgtgcgctttgcgaagagcatcttcattaacggtaacgtagtgactttgcattcggactcgatgatcttacatgatagcttacgcttactgccggggtctctggaaaagctctgtaaagattttggcctgaccgacaacgccaagaaagatctttccgaagtcatcaaagagcagggttacgcagtatacaagaaagacggtgtcacatttgacaagaagaaatcccttggcaattattttgagaacgtgcctgccgacgaccctacgctcaatgagtacttggagttcgattgtcgcagcctgtacgagattttgacgattgtgatggacatcgcaaatattggcctggaaaccttagtaatgtgcccgaccacagcgagcttagccatgcgtgtctataaagagcaataccgcgagcaatatgataaggtggccactcacttttatatgggcgagtggggtcaattcctcgaagagcacgttcgccaatcgtactacggtggtcgcactgaggtatttacccctcatttaccacatggttaccattacgatgttaactcgttgtacccgtatgtcatgaaaattgcaaagttcccggtagggtacccaaatttattgaaagacggccaggcagctaccaagtggaagcattggaagcgtcgtgcgatcgggggcggtgttatgtggtgtcgtgtggacgttcctgaagacatgtacatcccagtgctcccgaagcgtgacccgagcgggaagttattgttcccggttggtaagctcgagggagtgtggaccctgcctgagctcctggaagcggaaaagaatggctgtacgatcgaggcgatttaccagatggtatactgggagcatatggagccgatctttaaagaattcgttgagcactttgaagacctcaagaagaacagtaagggagcgaagcgcacctttgcaaagcttatccagaatagcttgtacgggaagttcggcatgaaccgcgttcgtgtgtcgttgggtgacatggaagaccgttacgacttgcatgagaagcagattccatataaagaattcaaacatgattgtaatggcttgacgcttgagttcatccaatatatctcggaaagcaaagcgagctatattcaaccgcacattgctacatacgtaacagcctatgctcgtatcctgttgtttcgtggtctgaaagaacaggctagcaagggcgtactgggctattgcgatactgactctattgccggtaccgccaaaatgccggacgaaatgatccatgacgaagattacggcaagtgggccttggaaggtgagctggaagaaggtatctttctccagccgaagttttacgcggaacgttacacgaacggcaaagaagtaattaaggccaaggggattccacgcgagaagatggaagagttaagtttcgagaactataaagagtggctcgagattatgaaagaaggccaacaagagcgcatcgacatctttgaaggttacgagagtcgcaagaagtttagcaccacactcaaggccagtgaagatttcgacacgttgcgtgagatgaagaagtctatcaatttactgctcgagcagaagcgcgacatcgactacaagggcaacgtgacacgtccacataagcgctatgactacggtggtggctcacatcaccaccatcatcat

SEQ ID NO: 20 - DNA, 1972 bp, Synthetic construct
  misc_feature 1..1972: note = APolTr-His-SET (nt)
  source 1..1972: mol_type = other DNA
ggctccaataagcaaaagaaagagcgccaaaagccggccaagcttctcaccttggacactgagacgcgcggcctcaccggtaatgtgttccgcgttggcctgtttgacgggacgaattattacaagtcgaatacattcgacgagatccttgacctgttcgagcaatataaagattacgaatgtcatgtatacgtacacaatttagacttcgacttggcgaaaatcgccaccactttgttcaagcgcgaccgtgtgcgctttgcgaagagcatcttcattaacggtaacgtagtgactttgcattcggactcgatgatcttacatgatagcttacgcttactgccggggtctctggaaaagctctgtaaagattttggcctgaccgacaacgccaagaaagatctttccgaagtcatcaaagagcagggttacgcagtatacaagaaagacggtgtcacatttgacaagaagaaatcccttggcaattattttgagaacgtgcctgccgacgaccctacgctcaatgagtacttggagttcgattgtcgcagcctgtacgagattttgacgattgtgatggacatcgcaaatattggcctggaaaccttagtaatgtgcccgaccacagcgagcttagccatgcgtgtctataaagagcaataccgcgagcaatatgataaggtggccactcacttttatatgggcgagtggggtcaattcctcgaagagcacgttcgccaatcgtactacggtggtcgcactgaggtatttacccctcatttaccacatggttaccattacgatgttaactcgttgtacccgtatgtcatgaaaattgcaaagttcccggtagggtacccaaatttattgaaagacggccaggcagctaccaagtggaagcattggaagcgtcgtgcgatcgggggcggtgttatgtggtgtcgtgtggacgttcctgaagacatgtacatcccagtgctcccgaagcgtgacccgagcgggaagttattgttcccggttggtaagctcgagggagtgtggaccctgcctgagctcctggaagcggaaaagaatggctgtacgatcgaggcgatttaccagatggtatactgggagcatatggagccgatctttaaagaattcgttgagcactttgaagacctcaagaagaacagtaagggagcgaagcgcacctttgcaaagcttatccagaatagcttgtacgggaagttcggcatgaaccgcgttcgtgtgtcgttgggtgacatggaagaccgttacgacttgcatgagaagcagattccatataaagaattcaaacatgattgtaatggcttgacgcttgagttcatccaatatatctcggaaagcaaagcgagctatattcaaccgcacattgctacatacgtaacagcctatgctcgtatcctgttgtttcgtggtctgaaagaacaggctagcaagggcgtactgggctattgcgatactgactctattgccggtaccgccaaaatgccggacgaaatgatccatgacgaagattacggcaagtgggccttggaaggtgagctggaagaaggtatctttctccagccgaagttttacgcggaacgttacacgaacggcaaagaagtaattaaggccaaggggattccacgcgagaagatggaagagttaagtttcgagaactataaagagtggctcgagattatgaaagaaggccaacaagagcgcatcgacatctttgaaggttacgagagtcgcaagaagtttagcaccacactcaaggccagtgaagatttcgacacgttgcgtgagatgaagaagtctatcaatttactgctcgagcagaagcgcgacatcgactacaagggcaacgtgacacgtccacataagcgctatgactacggtggtggctcacatcaccaccatcatcattcagaagaggacgaagagaaagaagaggacgggt

SEQ ID NO: 21 - DNA, 1911 bp, Synthetic construct
  misc_feature 1..1911: note = APolTr (nt)
  source 1..1911: mol_type = other DNA
ggctccaataagcaaaagaaagagcgccaaaagccggccaagcttctcaccttggacactgagacgcgcggcctcaccggtaatgtgttccgcgttggcctgtttgacgggacgaattattacaagtcgaatacattcgacgagatccttgacctgttcgagcaatataaagattacgaatgtcatgtatacgtacacaatttagacttcgacttggcgaaaatcgccaccactttgttcaagcgcgaccgtgtgcgctttgcgaagagcatcttcattaacggtaacgtagtgactttgcattcggactcgatgatcttacatgatagcttacgcttactgccggggtctctggaaaagctctgtaaagattttggcctgaccgacaacgccaagaaagatctttccgaagtcatcaaagagcagggttacgcagtatacaagaaagacggtgtcacatttgacaagaagaaatcccttggcaattattttgagaacgtgcctgccgacgaccctacgctcaatgagtacttggagttcgattgtcgcagcctgtacgagattttgacgattgtgatggacatcgcaaatattggcctggaaaccttagtaatgtgcccgaccacagcgagcttagccatgcgtgtctataaagagcaataccgcgagcaatatgataaggtggccactcacttttatatgggcgagtggggtcaattcctcgaagagcacgttcgccaatcgtactacggtggtcgcactgaggtatttacccctcatttaccacatggttaccattacgatgttaactcgttgtacccgtatgtcatgaaaattgcaaagttcccggtagggtacccaaatttattgaaagacggccaggcagctaccaagtggaagcattggaagcgtcgtgcgatcgggggcggtgttatgtggtgtcgtgtggacgttcctgaagacatgtacatcccagtgctcccgaagcgtgacccgagcgggaagttattgttcccggttggtaagctcgagggagtgtggaccctgcctgagctcctggaagcggaaaagaatggctgtacgatcgaggcgatttaccagatggtatactgggagcatatggagccgatctttaaagaattcgttgagcactttgaagacctcaagaagaacagtaagggagcgaagcgcacctttgcaaagcttatccagaatagcttgtacgggaagttcggcatgaaccgcgttcgtgtgtcgttgggtgacatggaagaccgttacgacttgcatgagaagcagattccatataaagaattcaaacatgattgtaatggcttgacgcttgagttcatccaatatatctcggaaagcaaagcgagctatattcaaccgcacattgctacatacgtaacagcctatgctcgtatcctgttgtttcgtggtctgaaagaacaggctagcaagggcgtactgggctattgcgatactgactctattgccggtaccgccaaaatgccggacgaaatgatccatgacgaagattacggcaagtgggccttggaaggtgagctggaagaaggtatctttctccagccgaagttttacgcggaacgttacacgaacggcaaagaagtaattaaggccaaggggattccacgcgagaagatggaagagttaagtttcgagaactataaagagtggctcgagattatgaaagaaggccaacaagagcgcatcgacatctttgaaggttacgagagtcgcaagaagtttagcaccacactcaaggccagtgaagatttcgacacgttgcgtgagatgaagaagtctatcaatttactgctcgagcagaagcgcgacatcgactacaagggcaacgtgacacgtccacataagcgctatgactacggt

SEQ ID NO: 22 - DNA, 1722 bp, Synthetic construct
  misc_feature 1..1722: note = Phi29 WT (nt)
  source 1..1722: mol_type = other DNA
aagcacatgccacgtaaaatgtatagctgtgattttgagactacgacgaaagttgaagattgccgtgtgtgggcgtatggttacatgaatattgaagatcactccgagtataagattggcaatagcctggatgaattcatggcgtgggtgctgaaggttcaggccgatttgtactttcataatctgaaatttgatggcgcttttatcattaactggctggagcgtaatggtttcaagtggagcgcagatggcctgccgaatacgtacaacaccattatcagccgtatgggccagtggtacatgatcgacatctgcctgggctataagggtaagcgtaagatccacaccgtgatttatgactccctgaaaaagctgccgtttccggtgaagaaaattgccaaagacttcaagctgacggttctgaagggcgacatcgattatcacaaggaacgtccggttggttacaagatcaccccggaagaatacgcgtacatcaaaaacgacattcaaatcatcgcagaggccttgctgattcagttcaagcaaggtctggaccgcatgactgccggtagcgattccctgaagggtttcaaagacattatcaccaccaaaaagttcaaaaaagtgttcccgacgctgagcctgggtctggataaagaggtccgttacgcttatcgtggcggcttcacctggttgaacgatcgtttcaaagaaaaagaaattggtgagggcatggtttttgatgttaactcactgtacccggcacaaatgtatagccgcctgctgccgtatggcgagccgatcgtgttcgagggtaaatacgtgtgggacgaagattacccgctgcatattcaacatatccgctgcgagttcgagctgaaggaaggctacatcccgaccattcagattaagcgtagccgtttttacaaaggtaatgaatacttgaagtcctcgggcggtgagattgcggatctgtggttaagcaacgtcgaccttgagctgatgaaagagcactatgacctctataacgttgagtacattagcggtctgaaattcaaagccacgacgggtctgtttaaagacttcattgacaagtggacctatatcaagacgacgagcgagggcgcgatcaaacagctggcgaagctgatgctgaattctctgtacggtaagtttgctagcaatccagatgtcaccggcaaagtgccgtatctgaaagaaaacggtgcgttgggttttcgcctgggtgaagaggaaaccaaagatccggtgtacaccccgatgggcgttttcattaccgcgtgggctcgttacaccacgattaccgcagcgcaggcatgttatgaccgtatcatttactgtgatacggatagcattcacttgaccggtaccgagatcccagatgtcatcaaagatattgtcgacccgaagaaactgggttactgggcccacgaaagcactttcaaacgcgcaaagtatctgcgtcagaaaacgtacatccaagacatttacatgaaagaggttgacggcaaattggtcgagggttcgccggacgactacaccgacatcaagttcagcgtgaagtgcgcgggtatgaccgacaaaatcaaaaaagaagtcacctttgagaactttaaggttggttttagccgcaagatgaagcctaaaccggttcaggtcccgggtggcgttgtgctggtcgacgacacctttactatcaag

SEQ ID NO: 23 - DNA, 18 bp, Synthetic construct
  misc_feature 1..18: note = 6x His tag (nt)
  source 1..18: mol_type = other DNA
catcaccaccatcatcat

SEQ ID NO: 24 - DNA, 34 bp, Synthetic construct
  misc_feature 1..34: note = SET tag (nt)
  source 1..34: mol_type = other DNA
tcagaagaggacgaagagaaagaagaggacgggt

SEQ ID NO: 25 - skipped

SEQ ID NO: 26 - protein, 98 aa, Synthetic construct
  REGION 1..98: note = SUMO tag (aa)
SDSEVNQEAKPEVKPEVKPETHINLKVSDGSSEIFFKIKKTTPLRRLMEAFAKRQGKEMDSLRFLYDGIRIQADQTPEDLDMEDNDIIEAHREQIGGS

SEQ ID NO: 27 - protein, 732 aa, Synthetic construct
  REGION 1..732: note = APol (aa)
MGSNKQKKERQKPAKLLTLDTETRGLTGNVFRVGLFDGTNYYKSNTFDEILDLFEQYKDYECHVYVHNLDFDLAKIATTLFKRDRVRFAKSIFINGNVVTLHSDSMILHDSLRLLPGSLEKLCKDFGLTDNAKKDLSEVIKEQGYAVYKKDGVTFDKKKSLGNYFENVPADDPTLNEYLEFDCRSLYEILTIVMDIANIGLETLVMCPTTASLAMRVYKEQYREQYDKVATHFYMGEWGQFLEEHVRQSYYGGRTEVFTPHLPHGYHYDVNSLYPYVMKIAKFPVGYPNLLKDGQAATKWKHWKRRAIGGGVMWCRVDVPEDMYIPVLPKRDPSGKLLFPVGKLEGVWTLPELLEAEKNGCTIEAIYQMVYWEHMEPIFKEFVEHFEDLKKNSKGAKRTFAKLIQNSLYGKFGMNRVRVSLGDMEDRYDLHEKQIPYKEFKHDCNGLTLEFIQYISESKASYIQPHIATYVTAYARILLFRGLKEQASKGVLGYCDTDSIAGTAKMPDEMIHDEDYGKWALEGELEEGIFLQPKFYAERYTNGKEVIKAKGIPREKMEELSFENYKEWLEIMKEGQQERIDIFEGYESRKKFSTTLKASEDFDTLREMKKSINLLLEQKRDIDYKGNVTRPHKRYDYGDKKDKIDYEDYKSREDKLNNMYDDVDDLKEQVDEIGYIKCMKQGDMYFEEYKHLTKSVKSKYFRRTGTPIDVWANESGWDVNELLEELRLMGVC

SEQ ID NO: 28 - protein, 741 aa, Synthetic construct
  REGION 1..741: note = APol-His (aa)
MGSNKQKKERQKPAKLLTLDTETRGLTGNVFRVGLFDGTNYYKSNTFDEILDLFEQYKDYECHVYVHNLDFDLAKIATTLFKRDRVRFAKSIFINGNVVTLHSDSMILHDSLRLLPGSLEKLCKDFGLTDNAKKDLSEVIKEQGYAVYKKDGVTFDKKKSLGNYFENVPADDPTLNEYLEFDCRSLYEILTIVMDIANIGLETLVMCPTTASLAMRVYKEQYREQYDKVATHFYMGEWGQFLEEHVRQSYYGGRTEVFTPHLPHGYHYDVNSLYPYVMKIAKFPVGYPNLLKDGQAATKWKHWKRRAIGGGVMWCRVDVPEDMYIPVLPKRDPSGKLLFPVGKLEGVWTLPELLEAEKNGCTIEAIYQMVYWEHMEPIFKEFVEHFEDLKKNSKGAKRTFAKLIQNSLYGKFGMNRVRVSLGDMEDRYDLHEKQIPYKEFKHDCNGLTLEFIQYISESKASYIQPHIATYVTAYARILLFRGLKEQASKGVLGYCDTDSIAGTAKMPDEMIHDEDYGKWALEGELEEGIFLQPKFYAERYTNGKEVIKAKGIPREKMEELSFENYKEWLEIMKEGQQERIDIFEGYESRKKFSTTLKASEDFDTLREMKKSINLLLEQKRDIDYKGNVTRPHKRYDYGDKKDKIDYEDYKSREDKLNNMYDDVDDLKEQVDEIGYIKCMKQGDMYFEEYKHLTKSVKSKYFRRTGTPIDVWANESGWDVNELLEELRLMGVCGGSHHHHHH

SEQ ID NO: 29 - protein, 647 aa, Synthetic construct
  REGION 1..647: note = APolTr-His (aa)
MGSNKQKKERQKPAKLLTLDTETRGLTGNVFRVGLFDGTNYYKSNTFDEILDLFEQYKDYECHVYVHNLDFDLAKIATTLFKRDRVRFAKSIFINGNVVTLHSDSMILHDSLRLLPGSLEKLCKDFGLTDNAKKDLSEVIKEQGYAVYKKDGVTFDKKKSLGNYFENVPADDPTLNEYLEFDCRSLYEILTIVMDIANIGLETLVMCPTTASLAMRVYKEQYREQYDKVATHFYMGEWGQFLEEHVRQSYYGGRTEVFTPHLPHGYHYDVNSLYPYVMKIAKFPVGYPNLLKDGQAATKWKHWKRRAIGGGVMWCRVDVPEDMYIPVLPKRDPSGKLLFPVGKLEGVWTLPELLEAEKNGCTIEAIYQMVYWEHMEPIFKEFVEHFEDLKKNSKGAKRTFAKLIQNSLYGKFGMNRVRVSLGDMEDRYDLHEKQIPYKEFKHDCNGLTLEFIQYISESKASYIQPHIATYVTAYARILLFRGLKEQASKGVLGYCDTDSIAGTAKMPDEMIHDEDYGKWALEGELEEGIFLQPKFYAERYTNGKEVIKAKGIPREKMEELSFENYKEWLEIMKEGQQERIDIFEGYESRKKFSTTLKASEDFDTLREMKKSINLLLEQKRDIDYKGNVTRPHKRYDYGGGSHHHHHH

SEQ ID NO: 30 - protein, 658 aa, Synthetic construct
  REGION 1..658: note = APolTr-His-SET (aa)
MGSNKQKKERQKPAKLLTLDTETRGLTGNVFRVGLFDGTNYYKSNTFDEILDLFEQYKDYECHVYVHNLDFDLAKIATTLFKRDRVRFAKSIFINGNVVTLHSDSMILHDSLRLLPGSLEKLCKDFGLTDNAKKDLSEVIKEQGYAVYKKDGVTFDKKKSLGNYFENVPADDPTLNEYLEFDCRSLYEILTIVMDIANIGLETLVMCPTTASLAMRVYKEQYREQYDKVATHFYMGEWGQFLEEHVRQSYYGGRTEVFTPHLPHGYHYDVNSLYPYVMKIAKFPVGYPNLLKDGQAATKWKHWKRRAIGGGVMWCRVDVPEDMYIPVLPKRDPSGKLLFPVGKLEGVWTLPELLEAEKNGCTIEAIYQMVYWEHMEPIFKEFVEHFEDLKKNSKGAKRTFAKLIQNSLYGKFGMNRVRVSLGDMEDRYDLHEKQIPYKEFKHDCNGLTLEFIQYISESKASYIQPHIATYVTAYARILLFRGLKEQASKGVLGYCDTDSIAGTAKMPDEMIHDEDYGKWALEGELEEGIFLQPKFYAERYTNGKEVIKAKGIPREKMEELSFENYKEWLEIMKEGQQERIDIFEGYESRKKFSTTLKASEDFDTLREMKKSINLLLEQKRDIDYKGNVTRPHKRYDYGGGSHHHHHHSEEDEEKEEDG

SEQ ID NO: 31 - protein, 575 aa, Synthetic construct [sequence omitted]

SEQ ID NO: 32 - protein, 638 aa, Synthetic construct
  REGION 1..638: note = APolTr (aa)
MGSNKQKKERQKPAKLLTLDTETRGLTGNVFRVGLFDGTNYYKSNTFDEILDLFEQYKDYECHVYVHNLDFDLAKIATTLFKRDRVRFAKSIFINGNVVTLHSDSMILHDSLRLLPGSLEKLCKDFGLTDNAKKDLSEVIKEQGYAVYKKDGVTFDKKKSLGNYFENVPADDPTLNEYLEFDCRSLYEILTIVMDIANIGLETLVMCPTTASLAMRVYKEQYREQYDKVATHFYMGEWGQFLEEHVRQSYYGGRTEVFTPHLPHGYHYDVNSLYPYVMKIAKFPVGYPNLLKDGQAATKWKHWKRRAIGGGVMWCRVDVPEDMYIPVLPKRDPSGKLLFPVGKLEGVWTLPELLEAEKNGCTIEAIYQMVYWEHMEPIFKEFVEHFEDLKKNSKGAKRTFAKLIQNSLYGKFGMNRVRVSLGDMEDRYDLHEKQIPYKEFKHDCNGLTLEFIQYISESKASYIQPHIATYVTAYARILLFRGLKEQASKGVLGYCDTDSIAGTAKMPDEMIHDEDYGKWALEGELEEGIFLQPKFYAERYTNGKEVIKAKGIPREKMEELSFENYKEWLEIMKEGQQERIDIFEGYESRKKFSTTLKASEDFDTLREMKKSINLLLEQKRDIDYKGNVTRPHKRYDYG

SEQ ID NO: 33 - protein, 2196 aa, Synthetic construct
  REGION 1..2196: note = APol (nt)
ATGGGCTCCAATAAGCAAAAGAAAGAGCGCCAAAAGCCGGCCAAGCTTCTCACCTTGGACACTGAGACGCGCGGCCTCACCGGTAATGTGTTCCGCGTTGGCCTGTTTGACGGGACGAATTATTACAAGTCGAATACATTCGACGAGATCCTTGACCTGTTCGAGCAATATAAAGATTACGAATGTCATGTATACGTACACAATTTAGACTTCGACTTGGCGAAAATCGCCACCACTTTGTTCAAGCGCGACCGTGTGCGCTTTGCGAAGAGCATCTTCATTAACGGTAACGTAGTGACTTTGCATTCGGACTCGATGATCTTACATGATAGCTTACGCTTACTGCCGGGGTCTCTGGAAAAGCTCTGTAAAGATTTTGGCCTGACCGACAACGCCAAGAAAGATCTTTCCGAAGTCATCAAAGAGCAGGGTTACGCAGTATACAAGAAAGACGGTGTCACATTTGACAAGAAGAAATCCCTTGGCAATTATTTTGAGAACGTGCCTGCCGACGACCCTACGCTCAATGAGTACTTGGAGTTCGATTGTCGCAGCCTGTACGAGATTTTGACGATTGTGATGGACATCGCAAATATTGGCCTGGAAACCTTAGTAATGTGCCCGACCACAGCGAGCTTAGCCATGCGTGTCTATAAAGAGCAATACCGCGAGCAATATGATAAGGTGGCCACTCACTTTTATATGGGCGAGTGGGGTCAATTCCTCGAAGAGCACGTTCGCCAATCGTACTACGGTGGTCGCACTGAGGTATTTACCCCTCATTTACCACATGGTTACCATTACGATGTTAACTCGTTGTACCCGTATGTCATGAAAATTGCAAAGTTCCCGGTAGGGTACCCAAATTTATTGAAAGACGGCCAGGCAGCTACCAAGTGGAAGCATTGGAAGCGTCGTGCGATCGGGGGCGGTGTTATGTGGTGTCGTGTGGACGTTCCTGAAGACATGTACATCCCAGTGCTCCCGAAGCGTGACCCGAGCGGGAAGTTATTGTTCCCGGTTGGTAAGCTCGAGGGAGTGTGGACCCTGCCTGAGCTCCTGGAAGCGGAAAAGAATGGCTGTACGATCGAGGCGATTTACCAGATGGTATACTGGGAGCATATGGAGCCGATCTTTAAAGAATTCGTTGAGCACTTTGAAGACCTCAAGAAGAACAGTAAGGGAGCGAAGCGCACCTTTGCAAAGCTTATCCAGAATAGCTTGTACGGGAAGTTCGGCATGAACCGCGTTCGTGTGTCGTTGGGTGACATGGAAGACCGTTACGACTTGCATGAGAAGCAGATTCCATATAAAGAATTCAAACATGATTGTAATGGCTTGACGCTTGAGTTCATCCAATATATCTCGGAAAGCAAAGCGAGCTATATTCAACCGCACATTGCTACATACGTAACAGCCTATGCTCGTATCCTGTTGTTTCGTGGTCTGAAAGAACAGGCTAGCAAGGGCGTACTGGGCTATTGCGATACTGACTCTATTGCCGGTACCGCCAAAATGCCGGACGAAATGATCCATGACGAAGATTACGGCAAGTGGGCCTTGGAAGGTGAGCTGGAAGAAGGTATCTTTCTCCAGCCGAAGTTTTACGCGGAACGTTACACGAACGGCAAAGAAGTAATTAAGGCCAAGGGGATTCCACGCGAGAAGATGGAAGAGTTAAGTTTCGAGAACTATAAAGAGTGGCTCGAGATTATGAAAGAAGGCCAACAAGAGCGCATCGACATCTTTGAAGGTTACGAGAGTCGCAAGAAGTTTAGCACCACACTCAAGGCCAGTGAAGATTTCGACACGTTGCGTGAGATGAAGAAGTCTATCAATTTACTGCTCGAGCAGAAGCGCGACATCGACTACAAGGGCAACGTGACACGTCCACATAAGCGCTATGACTACGGTGATAAGAAAGACAAGATCGATTATGAAGACTATAAGAGCCGTGAAGACAAGTTAAACAACATGTACGACGATGTAGACGACTTAAAAGAGCAAGTTGACGAGATCGGCTACATCAAGTGCATGAAGCAAGGCGATATGTATTTTGAAGAGTACAAACATCTTACGAAGTCTGTGAAAAGTAAGTATTTCCGCCGCACTGGCACCCCAATCGACGTATGGGCGAACGAATCCGGTTGGGACGTAAACGAGTTATTAGAAGAGCTTCGTCTGATGGGCGTGTGC

SEQ ID NO: 34 - DNA, 2223 bp, Synthetic construct
  misc_feature 1..2223: note = APol-His (nt)
  source 1..2223: mol_type = other DNA
atgggctccaataagcaaaagaaagagcgccaaaagccggccaagcttctcaccttggacactgagacgcgcggcctcaccggtaatgtgttccgcgttggcctgtttgacgggacgaattattacaagtcgaatacattcgacgagatccttgacctgttcgagcaatataaagattacgaatgtcatgtatacgtacacaatttagacttcgacttggcgaaaatcgccaccactttgttcaagcgcgaccgtgtgcgctttgcgaagagcatcttcattaacggtaacgtagtgactttgcattcggactcgatgatcttacatgatagcttacgcttactgccggggtctctggaaaagctctgtaaagattttggcctgaccgacaacgccaagaaagatctttccgaagtcatcaaagagcagggttacgcagtatacaagaaagacggtgtcacatttgacaagaagaaatcccttggcaattattttgagaacgtgcctgccgacgaccctacgctcaatgagtacttggagttcgattgtcgcagcctgtacgagattttgacgattgtgatggacatcgcaaatattggcctggaaaccttagtaatgtgcccgaccacagcgagcttagccatgcgtgtctataaagagcaataccgcgagcaatatgataaggtggccactcacttttatatgggcgagtggggtcaattcctcgaagagcacgttcgccaatcgtactacggtggtcgcactgaggtatttacccctcatttaccacatggttaccattacgatgttaactcgttgtacccgtatgtcatgaaaattgcaaagttcccggtagggtacccaaatttattgaaagacggccaggcagctaccaagtggaagcattggaagcgtcgtgcgatcgggggcggtgttatgtggtgtcgtgtggacgttcctgaagacatgtacatcccagtgctcccgaagcgtgacccgagcgggaagttattgttcccggttggtaagctcgagggagtgtggaccctgcctgagctcctggaagcggaaaagaatggctgtacgatcgaggcgatttaccagatggtatactgggagcatatggagccgatctttaaagaattcgttgagcactttgaagacctcaagaagaacagtaagggagcgaagcgcacctttgcaaagcttatccagaatagcttgtacgggaagttcggcatgaaccgcgttcgtgtgtcgttgggtgacatggaagaccgttacgacttgcatgagaagcagattccatataaagaattcaaacatgattgtaatggcttgacgcttgagttcatccaatatatctcggaaagcaaagcgagctatattcaaccgcacattgctacatacgtaacagcctatgctcgtatcctgttgtttcgtggtctgaaagaacaggctagcaagggcgtactgggctattgcgatactgactctattgccggtaccgccaaaatgccggacgaaatgatccatgacgaagattacggcaagtgggccttggaaggtgagctggaagaaggtatctttctccagccgaagttttacgcggaacgttacacgaacggcaaagaagtaattaaggccaaggggattccacgcgagaagatggaagagttaagtttcgagaactataaagagtggctcgagattatgaaagaaggccaacaagagcgcatcgacatctttgaaggttacgagagtcgcaagaagtttagcaccacactcaaggccagtgaagatttcgacacgttgcgtgagatgaagaagtctatcaatttactgctcgagcagaagcgcgacatcgactacaagggcaacgtgacacgtccacataagcgctatgactacggtgataagaaagacaagatcgattatgaagactataagagccgtgaagacaagttaaacaacatgtacgacgatgtagacgacttaaaagagcaagttgacgagatcggctacatcaagtgcatgaagcaaggcgatatgtattttgaagagtacaaacatcttacgaagtctgtgaaaagtaagtatttccgccgcactggcaccccaatcgacgtatgggcgaacgaatccggttgggacgtaaacgagttattagaagagcttcgtctgatgggcgtgtgcggtggctcacatcaccaccatcatcat

SEQ ID NO: 35 - DNA, 1941 bp, Synthetic construct
  misc_feature 1..1941: note = APolTr-His (nt)
  source 1..1941: mol_type = other DNA
atgggctccaataagcaaaagaaagagcgccaaaagccggccaagcttctcaccttggacactgagacgcgcggcctcaccggtaatgtgttccgcgttggcctgtttgacgggacgaattattacaagtcgaatacattcgacgagatccttgacctgttcgagcaatataaagattacgaatgtcatgtatacgtacacaatttagacttcgacttggcgaaaatcgccaccactttgttcaagcgcgaccgtgtgcgctttgcgaagagcatcttcattaacggtaacgtagtgactttgcattcggactcgatgatcttacatgatagcttacgcttactgccggggtctctggaaaagctctgtaaagattttggcctgaccgacaacgccaagaaagatctttccgaagtcatcaaagagcagggttacgcagtatacaagaaagacggtgtcacatttgacaagaagaaatcccttggcaattattttgagaacgtgcctgccgacgaccctacgctcaatgagtacttggagttcgattgtcgcagcctgtacgagattttgacgattgtgatggacatcgcaaatattggcctggaaaccttagtaatgtgcccgaccacagcgagcttagccatgcgtgtctataaagagcaataccgcgagcaatatgataaggtggccactcacttttatatgggcgagtggggtcaattcctcgaagagcacgttcgccaatcgtactacggtggtcgcactgaggtatttacccctcatttaccacatggttaccattacgatgttaactcgttgtacccgtatgtcatgaaaattgcaaagttcccggtagggtacccaaatttattgaaagacggccaggcagctaccaagtggaagcattggaagcgtcgtgcgatcgggggcggtgttatgtggtgtcgtgtggacgttcctgaagacatgtacatcccagtgctcccgaagcgtgacccgagcgggaagttattgttcccggttggtaagctcgagggagtgtggaccctgcctgagctcctggaagcggaaaagaatggctgtacgatcgaggcgatttaccagatggtatactgggagcatatggagccgatctttaaagaattcgttgagcactttgaagacctcaagaagaacagtaagggagcgaagcgcacctttgcaaagcttatccagaatagcttgtacgggaagttcggcatgaaccgcgttcgtgtgtcgttgggtgacatggaagaccgttacgacttgcatgagaagcagattccatataaagaattcaaacatgattgtaatggcttgacgcttgagttcatccaatatatctcggaaagcaaagcgagctatattcaaccgcacattgctacatacgtaacagcctatgctcgtatcctgttgtttcgtggtctgaaagaacaggctagcaagggcgtactgggctattgcgatactgactctattgccggtaccgccaaaatgccggacgaaatgatccatgacgaagattacggcaagtgggccttggaaggtgagctggaagaaggtatctttctccagccgaagttttacgcggaacgttacacgaacggcaaagaagtaattaaggccaaggggattccacgcgagaagatggaagagttaagtttcgagaactataaagagtggctcgagattatgaaagaaggccaacaagagcgcatcgacatctttgaaggttacgagagtcgcaagaagtttagcaccacactcaaggccagtgaagatttcgacacgttgcgtgagatgaagaagtctatcaatttactgctcgagcagaagcgcgacatcgactacaagggcaacgtgacacgtccacataagcgctatgactacggtggtggctcacatcaccaccatcatcat

SEQ ID NO: 36 - DNA, 1975 bp, Synthetic construct
  misc_feature 1..1975: note = APolTr-His-SET (nt)
  source 1..1975: mol_type = other DNA
atgggctccaataagcaaaagaaagagcgccaaaagccggccaagcttctcaccttggacactgagacgcgcggcctcaccggtaatgtgttccgcgttggcctgtttgacgggacgaattattacaagtcgaatacattcgacgagatccttgacctgttcgagcaatataaagattacgaatgtcatgtatacgtacacaatttagacttcgacttggcgaaaatcgccaccactttgttcaagcgcgaccgtgtgcgctttgcgaagagcatcttcattaacggtaacgtagtgactttgcattcggactcgatgatcttacatgatagcttacgcttactgccggggtctctggaaaagctctgtaaagattttggcctgaccgacaacgccaagaaagatctttccgaagtcatcaaagagcagggttacgcagtatacaagaaagacggtgtcacatttgacaagaagaaatcccttggcaattattttgagaacgtgcctgccgacgaccctacgctcaatgagtacttggagttcgattgtcgcagcctgtacgagattttgacgattgtgatggacatcgcaaatattggcctggaaaccttagtaatgtgcccgaccacagcgagcttagccatgcgtgtctataaagagcaataccgcgagcaatatgataaggtggccactcacttttatatgggcgagtggggtcaattcctcgaagagcacgttcgccaatcgtactacggtggtcgcactgaggtatttacccctcatttaccacatggttaccattacgatgttaactcgttgtacccgtatgtcatgaaaattgcaaagttcccggtagggtacccaaatttattgaaagacggccaggcagctaccaagtggaagcattggaagcgtcgtgcgatcgggggcggtgttatgtggtgtcgtgtggacgttcctgaagacatgtacatcccagtgctcccgaagcgtgacccgagcgggaagttattgttcccggttggtaagctcgagggagtgtggaccctgcctgagctcctggaagcggaaaagaatggctgtacgatcgaggcgatttaccagatggtatactgggagcatatggagccgatctttaaagaattcgttgagcactttgaagacctcaagaagaacagtaagggagcgaagcgcacctttgcaaagcttatccagaatagcttgtacgggaagttcggcatgaaccgcgttcgtgtgtcgttgggtgacatggaagaccgttacgacttgcatgagaagcagattccatataaagaattcaaacatgattgtaatggcttgacgcttgagttcatccaatatatctcggaaagcaaagcgagctatattcaaccgcacattgctacatacgtaacagcctatgctcgtatcctgttgtttcgtggtctgaaagaacaggctagcaagggcgtactgggctattgcgatactgactctattgccggtaccgccaaaatgccggacgaaatgatccatgacgaagattacggcaagtgggccttggaaggtgagctggaagaaggtatctttctccagccgaagttttacgcggaacgttacacgaacggcaaagaagtaattaaggccaaggggattccacgcgagaagatggaagagttaagtttcgagaactataaagagtggctcgagattatgaaagaaggccaacaagagcgcatcgacatctttgaaggttacgagagtcgcaagaagtttagcaccacactcaaggccagtgaagatttcgacacgttgcgtgagatgaagaagtctatcaatttactgctcgagcagaagcgcgacatcgactacaagggcaacgtgacacgtccacataagcgctatgactacggtggtggctcacatcaccaccatcatcattcagaagaggacgaagagaaagaagaggacgggt

SEQ ID NO: 37 - DNA, 1914 bp, Synthetic construct
  misc_feature 1..1914: note = APolTr (nt)
  source 1..1914: mol_type = other DNA
atgggctccaataagcaaaagaaagagcgccaaaagccggccaagcttctcaccttggacactgagacgcgcggcctcaccggtaatgtgttccgcgttggcctgtttgacgggacgaattattacaagtcgaatacattcgacgagatccttgacctgttcgagcaatataaagattacgaatgtcatgtatacgtacacaatttagacttcgacttggcgaaaatcgccaccactttgttcaagcgcgaccgtgtgcgctttgcgaagagcatcttcattaacggtaacgtagtgactttgcattcggactcgatgatcttacatgatagcttacgcttactgccggggtctctggaaaagctctgtaaagattttggcctgaccgacaacgccaagaaagatctttccgaagtcatcaaagagcagggttacgcagtatacaagaaagacggtgtcacatttgacaagaagaaatcccttggcaattattttgagaacgtgcctgccgacgaccctacgctcaatgagtacttggagttcgattgtcgcagcctgtacgagattttgacgattgtgatggacatcgcaaatattggcctggaaaccttagtaatgtgcccgaccacagcgagcttagccatgcgtgtctataaagagcaataccgcgagcaatatgataaggtggccactcacttttatatgggcgagtggggtcaattcctcgaagagcacgttcgccaatcgtactacggtggtcgcactgaggtatttacccctcatttaccacatggttaccattacgatgttaactcgttgtacccgtatgtcatgaaaattgcaaagttcccggtagggtacccaaatttattgaaagacggccaggcagctaccaagtggaagcattggaagcgtcgtgcgatcgggggcggtgttatgtggtgtcgtgtggacgttcctgaagacatgtacatcccagtgctcccgaagcgtgacccgagcgggaagttattgttcccggttggtaagctcgagggagtgtggaccctgcctgagctcctggaagcggaaaagaatggctgtacgatcgaggcgatttaccagatggtatactgggagcatatggagccgatctttaaagaattcgttgagcactttgaagacctcaagaagaacagtaagggagcgaagcgcacctttgcaaagcttatccagaatagcttgtacgggaagttcggcatgaaccgcgttcgtgtgtcgttgggtgacatggaagaccgttacgacttgcatgagaagcagattccatataaagaattcaaacatgattgtaatggcttgacgcttgagttcatccaatatatctcggaaagcaaagcgagctatattcaaccgcacattgctacatacgtaacagcctatgctcgtatcctgttgtttcgtggtctgaaagaacaggctagcaagggcgtactgggctattgcgatactgactctattgccggtaccgccaaaatgccggacgaaatgatccatgacgaagattacggcaagtgggccttggaaggtgagctggaagaaggtatctttctccagccgaagttttacgcggaacgttacacgaacggcaaagaagtaattaaggccaaggggattccacgcgagaagatggaagagttaagtttcgagaactataaagagtggctcgagattatgaaagaaggccaacaagagcgcatcgacatctttgaaggttacgagagtcgcaagaagtttagcaccacactcaaggccagtgaagatttcgacacgttgcgtgagatgaagaagtctatcaatttactgctcgagcagaagcgcgacatcgactacaagggcaacgtgacacgtccacataagcgctatgactacggt

SEQ ID NO: 38 - DNA, 1725 bp, Synthetic construct
  misc_feature 1..1725: note = Phi29 WT (nt)
  source 1..1725: mol_type = other DNA
atgaagcacatgccacgtaaaatgtatagctgtgattttgagactacgacgaaagttgaagattgccgtgtgtgggcgtatggttacatgaatattgaagatcactccgagtataagattggcaatagcctggatgaattcatggcgtgggtgctgaaggttcaggccgatttgtactttcataatctgaaatttgatggcgcttttatcattaactggctggagcgtaatggtttcaagtggagcgcagatggcctgccgaatacgtacaacaccattatcagccgtatgggccagtggtacatgatcgacatctgcctgggctataagggtaagcgtaagatccacaccgtgatttatgactccctgaaaaagctgccgtttccggtgaagaaaattgccaaagacttcaagctgacggttctgaagggcgacatcgattatcacaaggaacgtccggttggttacaagatcaccccggaagaatacgcgtacatcaaaaacgacattcaaatcatcgcagaggccttgctgattcagttcaagcaaggtctggaccgcatgactgccggtagcgattccctgaagggtttcaaagacattatcaccaccaaaaagttcaaaaaagtgttcccgacgctgagcctgggtctggataaagaggtccgttacgcttatcgtggcggcttcacctggttgaacgatcgtttcaaagaaaaagaaattggtgagggcatggtttttgatgttaactcactgtacccggcacaaatgtatagccgcctgctgccgtatggcgagccgatcgtgttcgagggtaaatacgtgtgggacgaagattacccgctgcatattcaacatatccgctgcgagttcgagctgaaggaaggctacatcccgaccattcagattaagcgtagccgtttttacaaaggtaatgaatacttgaagtcctcgggcggtgagattgcggatctgtggttaagcaacgtcgaccttgagctgatgaaagagcactatgacctctataacgttgagtacattagcggtctgaaattcaaagccacgacgggtctgtttaaagacttcattgacaagtggacctatatcaagacgacgagcgagggcgcgatcaaacagctggcgaagctgatgctgaattctctgtacggtaagtttgctagcaatccagatgtcaccggcaaagtgccgtatctgaaagaaaacggtgcgttgggttttcgcctgggtgaagaggaaaccaaagatccggtgtacaccccgatgggcgttttcattaccgcgtgggctcgttacaccacgattaccgcagcgcaggcatgttatgaccgtatcatttactgtgatacggatagcattcacttgaccggtaccgagatcccagatgtcatcaaagatattgtcgacccgaagaaactgggttactgggcccacgaaagcactttcaaacgcgcaaagtatctgcgtcagaaaacgtacatccaagacatttacatgaaagaggttgacggcaaattggtcgagggttcgccggacgactacaccgacatcaagttcagcgtgaagtgcgcgggtatgaccgacaaaatcaaaaaagaagtcacctttgagaactttaaggttggttttagccgcaagatgaagcctaaaccggttcaggtcccgggtggcgttgtgctggtcgacgacacctttactatcaag